European Patent Application EP 4 635 976 A1, published October 22, 2025. Title: UNI-TABS specific antibody. Applicant: MEDIGENE IMMUNOTHERAPIES GMBH. Application EP. The sequence listing filed with the application follows.

SEQUENCE LISTING (163 sequences)

SEQ ID NO: 1 - protein, 20 aa, synthetic construct
VHSGVSTDPQPLKEQPALND

SEQ ID NO: 2 - protein, 20 aa, synthetic construct
NGKEVHSGVSTDPQPLKEQP

SEQ ID NO: 3 - protein, 20 aa, unidentified
GKEVHSGVSTDPQPLKEQPA

SEQ ID NO: 4 - protein, 20 aa, synthetic construct
KEVHSGVSTDPQPLKEQPAL

SEQ ID NO: 5 - protein, 20 aa, synthetic construct
SRYCLSSRLRVSATFWQNPR

SEQ ID NO: 6 - protein, 20 aa, synthetic construct
ALNDSRYCLSSRLRVSATFW

SEQ ID NO: 7 - protein, 20 aa, synthetic construct
LNDSRYCLSSRLRVSATFWQ

SEQ ID NO: 8 - protein, 20 aa, synthetic construct
NDSRYCLSSRLRVSATFWQN

SEQ ID NO: 9 - protein, 20 aa, synthetic construct
QNPRNHFRCQVQFYGLSEND

SEQ ID NO: 10 - protein, 20 aa, synthetic construct
PRNHFRCQVQFYGLSENDEW

SEQ ID NO: 11 - protein, 20 aa, synthetic construct
RCQVQFYGLSENDEWTQDRA

SEQ ID NO: 12 - protein, 20 aa, synthetic construct
EWTQDRAKPVTQIVSAEAWG

SEQ ID NO: 13 - protein, 20 aa, synthetic construct
TQDRAKPVTQIVSAEAWGRA

SEQ ID NO: 14 - protein, 20 aa, synthetic construct
KPVTQIVSAEAWGRADCGIT

SEQ ID NO: 15 - protein, 20 aa, synthetic construct
AVAWSNKSDFACANAFNNSI

SEQ ID NO: 16 - protein, 20 aa, synthetic construct
AWSNKSDFACANAFNNSIIP

SEQ ID NO: 17 - protein, 20 aa, synthetic construct
SNKSDFACANAFNNSIIPED

SEQ ID NO: 18 - protein, 20 aa, synthetic construct
IPEDTFFPSSDVPCDVKLVE

SEQ ID NO: 19 - protein, 20 aa, synthetic construct
EDTFFPSSDVPCDVKLVEKS

SEQ ID NO: 20 - protein, 20 aa, synthetic construct
TFFPSSDVPCDVKLVEKSFE

SEQ ID NO: 21 - protein, 20 aa, synthetic construct
GKEVHSGVCTDPQPLKEQPA

SEQ ID NO: 22 - protein, 20 aa, synthetic construct
RCQVQFYGLSENDEWTQDRA

SEQ ID NO: 23 - protein, 20 aa, synthetic construct
LNDSRYCLSSRLRVSATFWQ

SEQ ID NO: 24 - protein, 20 aa, synthetic construct
KPVTQIVSAEAWGRADCGIT

SEQ ID NO: 25 - protein, 6 aa, synthetic construct
  VARIANT 5: note = X may be A, R, N, D, C, Q, E, G, H, I, L, K, M, F, P, S, T, W, Y, V
EVPKXR

SEQ ID NO: 26 - protein, 9 aa, synthetic construct
  VARIANT 6: note = X may be A, R, N, D, C, Q, E, G, H, I, L, K, M, F, P, S, T, TW, Y, V
GEVPKXRFS

SEQ ID NO: 27 - protein, 12 aa, synthetic construct
  VARIANT 1: note = X is selected from D and E
  VARIANT 2: note = X is selected from K, R, H
  VARIANT 8: note = X is selected from A, R, N, D, C, Q, E, G, H, I, L, K, M, F, P, S, T, W, Y, V
  VARIANT 12: note = X is selected from G, L, A, V, M, I, S, T
XXGEVPKXRFSX

SEQ ID NO: 28 - protein, 12 aa, synthetic construct
  VARIANT 2: note = X is selected from K, R, H
  VARIANT 8: note = X is selected from A, R, N, D, C, Q, E, G, H, I, L, K, M, F, P, S, T, W, Y, V
  VARIANT 12: note = X is selected from G, L, A, V, M, I, S, T
DXGEVPKXRFSX

SEQ ID NO: 29 - protein, 12 aa, synthetic construct
  VARIANT 2: note = X is seleceted from K, R, and H
  VARIANT 8: note = X is selected from A, R, N, D, C, Q, E, G, H, I, L, K, M, F, P, S, T, W, Y, V
  VARIANT 12: note = X is selected from G, L, A, V, M, I, S, and T
EXGEVPKXRFSX

SEQ ID NO: 30 - protein, 12 aa, synthetic construct
  VARIANT 1: note = X is selected from D and E
  VARIANT 8: note = X is selected from A, R, N, D, C, Q, E, G, H, I, L, K, M, F, P, S, T, W, Y, V
  VARIANT 12: note = X is selected from G, L, A, V, M, I, S, and T
XKGEVPKXRFSX

SEQ ID NO: 31 - protein, 12 aa, synthetic construct
  VARIANT 1: note = X is selected from D and E
  VARIANT 8: note = X is selected from A, R, N, D, C, Q, E, G, H, I, L, K, M, F, P, S, T, W, Y, V
  VARIANT 12: note = X is selected from G, L, A, V, M, I, S, and T
XRGEVPKXRFSX

SEQ ID NO: 32 - protein, 12 aa, synthetic construct
  VARIANT 1: note = X is selected from D and E
  VARIANT 8: note = X is selected from A, R, N, D, C, Q, E, G, H, I, L, K, M, F, P, S, T, W, Y, V
  VARIANT 12: note = X is selected from G, L, A, V, M, I, S, and T
XHGEVPKXRFSX

SEQ ID NO: 33 - protein, 12 aa, synthetic construct
  VARIANT 1: note = X is selected from D and E
  VARIANT 2: note = X is selected from K, R, and H
  VARIANT 8: note = X is selected from A, R, N, D, C, Q, E, G, H, I, L, K, M, F, P, S, T, W, Y, V
XXGEVPKXRFSG

SEQ ID NO: 34 - protein, 12 aa, synthetic construct
  VARIANT 1: note = X is selected from D and E
  VARIANT 2: note = X is selected from K, R, and H
  VARIANT 8: note = X is selected from A, R, N, D, C, Q, E, G, H, I, L, K, M, F, P, S, T, W, Y, V
XXGEVPKXRFSL

SEQ ID NO: 35 - protein, 12 aa, synthetic construct
  VARIANT 1: note = X is selected from D and E
  VARIANT 2: note = X is selected from K, R, and H
  VARIANT 8: note = X is selected from A, R, N, D, C, Q, E, G, H, I, L, K, M, F, P, S, T, W, Y, V
XXGEVPKXRFSA

SEQ ID NO: 36 - protein, 12 aa, synthetic construct
  VARIANT 1: note = X is selected from D and E
  VARIANT 2: note = X is selected from K, R, and H
  VARIANT 8: note = X is selected from A, R, N, D, C, Q, E, G, H, I, L, K, M, F, P, S, T, W, Y, V
XXGEVPKXRFSV

SEQ ID NO: 37 - protein, 12 aa, synthetic construct
  VARIANT 1: note = X is selected from D and E
  VARIANT 2: note = X is selected from K, R, and H
  VARIANT 8: note = X is selected from A, R, N, D, C, Q, E, G, H, I, L, K, M, F, P, S, T, W, Y, V
XXGEVPKXRFSM

SEQ ID NO: 38 - protein, 12 aa, synthetic construct
  VARIANT 1: note = X is selected from D and E
  VARIANT 2: note = X is selected from K, R, and H
  VARIANT 8: note = X is selected from A, R, N, D, C, Q, E, G, H, I, L, K, M, F, P, S, T, W, Y, V
XXGEVPKXRFSI

SEQ ID NO: 39 - protein, 12 aa, synthetic construct
  VARIANT 1: note = X is selected from D and E
  VARIANT 2: note = X is selected from K, R, and H
  VARIANT 8: note = X is is selected from A, R, N, D, C, Q, E, G, H, I, L, K, M, F, P, S, T, W, Y, V
XXGEVPKXRFSS

SEQ ID NO: 40 - protein, 12 aa, synthetic construct
  VARIANT 1: note = X is selected from D and E
  VARIANT 2: note = X is selected from K, R, and H
  VARIANT 8: note = X is selected from A, R, N, D, C, Q, E, G, H, I, L, K, M, F, P, S, T, W, Y, V
XXGEVPKXRFST

SEQ ID NO: 41 - protein, 12 aa, synthetic construct
  VARIANT 8: note = X is selected from A, R, N, D, C, Q, E, G, H, I, L, K, M, F, P, S, T, W, Y, V
  VARIANT 12: note = X is selected from G, L, A, V, M, I, S, and T
DKGEVPKXRFSX

SEQ ID NO: 42 - protein, 12 aa, synthetic construct
  VARIANT 8: note = X is selected from A, R, N, D, C, Q, E, G, H, I, L, K, M, F, P, S, T, W, Y, V
  VARIANT 12: note = X is selected from G, L, A, V, M, I, S, and T
DRGEVPKXRFSX

SEQ ID NO: 43 - protein, 12 aa, synthetic construct
  VARIANT 8: note = X is selected from A, R, N, D, C, Q, E, G, H, I, L, K, M, F, P, S, T, W, Y, V
  VARIANT 12: note = X is selected from G, L, A, V, M, I, S, and T
DHGEVPKXRFSX

SEQ ID NO: 44 - protein, 12 aa, synthetic construct
  VARIANT 8: note = X is selected from A, R, N, D, C, Q, E, G, H, I, L, K, M, F, P, S, T, W, Y, V
  VARIANT 12: note = X is selected from G, L, A, V, M, I, S, and T
EKGEVPKXRFSX

SEQ ID NO: 45 - protein, 12 aa, synthetic construct
  VARIANT 8: note = X is selected from A, R, N, D, C, Q, E, G, H, I, L, K, M, F, P, S, T, W, Y, V
  VARIANT 12: note = X is selected from G, L, A, V, M, I, S, and T
ERGEVPKXRFSX

SEQ ID NO: 46 - protein, 12 aa, synthetic construct
  VARIANT 8: note = X is selected from A, R, N, D, C, Q, E, G, H, I, L, K, M, F, P, S, T, W, Y, V
  VARIANT 12: note = X is selected from G, L, A, V, M, I, S, and T
EHGEVPKXRFSX

SEQ ID NO: 47 - protein, 12 aa, synthetic construct
DKGEVPKDRFSA

SEQ ID NO: 48 - protein, 11 aa, synthetic construct
KGEVPKDRFSA

SEQ ID NO: 49 - protein, 10 aa, synthetic construct
GEVPKDRFSA

SEQ ID NO: 50 - protein, 9 aa, synthetic construct
GEVPKDRFS

SEQ ID NO: 51 - protein, 11 aa, synthetic construct
DKGEVPKDRFS

SEQ ID NO: 52 - protein, 9 aa, synthetic construct
KGEVPKDRF

SEQ ID NO: 53 - protein, 9 aa, synthetic construct
YPYDVPDYA

SEQ ID NO: 54 - protein, 18 aa, synthetic construct
GSGDKGEVPKDRFSAGSG

SEQ ID NO: 55 - protein, 17 aa, synthetic construct
GSGKGEVPKDRFSAGSG

SEQ ID NO: 56 - protein, 16 aa, synthetic construct
GSGGEVPKDRFSAGSG

SEQ ID NO: 57 - protein, 15 aa, synthetic construct
GSGGEVPKDRFSGSG

SEQ ID NO: 58 - protein, 17 aa, synthetic construct
GSGDKGEVPKDRFSGSG

SEQ ID NO: 59 - protein, 15 aa, synthetic construct
GSGKGEVPKDRFGSG

SEQ ID NO: 60 - protein, 15 aa, synthetic construct
GSGYPYDVPDYAGSG

SEQ ID NO: 61-63 - skipped (3 entries)

SEQ ID NO: 64 - protein, 129 aa, synthetic construct
MKSLRVLLVILWLQLSWVWSQQKEVEQNSGPLSVPEGAIASLNCTYSDRGSQSFFWYRQYSGKSPELIMFIYSNGDKEDGRFTAQLNKASQYVSLLIRDSQPSDSATYLCAADDKIIFGKGTRLHILPN

SEQ ID NO: 65 - protein, 134 aa, synthetic construct
MEKMLECAFIVLWLQLGWLSGEDQVTQSPEALRLQEGESSSLNCSYTVSGLRGLFWYRQDPGKGPEFLFTLYSAGEEKEKERLKATLTKKESFLHITAPKPEDSATYLCAVHSTAQAGTALIFGKGTTLSVSSN

SEQ ID NO: 66 - protein, 128 aa, synthetic construct
MWGVFLLYVSMKMGGTTGQNIDQPTEMTATEGAIVQINCTYQTSGFNGLFWYQQHAGEAPTFLSYNVLDGLEEKGRFSSFLSRSKGYSYLLLKELQMKDSASYLCAVRGDSSYKLIFGSGTRLLVRPD

SEQ ID NO: 67 - protein, 140 aa, synthetic construct
IQNPDPAVYQLRDSKSSDKSVCLFTDFDSQTNVSQSKDSDVYITDKTVLDMRSMDFKSNSAVAWSNKSDFACANAFNNSIIPEDTFFPSSDVPCDVKLVEKSFETDTNLNFQNLSVIGFRILLLKVAGFNLLMTLRLWSS

SEQ ID NO: 68 - protein, 140 aa, synthetic construct
IQNPDPAVYQLRDSKSSDKSVCLFTDFDSQTNVSQSKDSDVYITDKCVLDMRSMDFKSNSAVAWSNKSDFACANAFNNSIIPEDTFFPSSDVPCDVKLVEKSFETDTNLNFQNLSVIGFRILLLKVAGFNLLMTLRLWSS

SEQ ID NO: 69 - protein, 140 aa, synthetic construct; identical to SEQ ID NO: 68

SEQ ID NO: 70 - protein, 131 aa, synthetic construct
MGSWTLCCVSLCILVAKHTDAGVIQSPRHEVTEMGQEVTLRCKPISGHDYLFWYRQTMMRGLELLIYFNNNVPIDDSGMPEDRFSAKMPNASFSTLKIQPSEPRDSAVYFCASSRGGSGYTFGSGTRLTVV

SEQ ID NO: 71 - protein, 134 aa, synthetic construct
MGFRLLCCVAFCLLGAGPVDSGVTQTPKHLITATGQRVTLRCSPRSGDLSVYWYQQSLDQGLQFLIQYYNGEERAKGNILERFSAQQFPDLHSELNLSSLELGDSALYFCASSTHRGQTNYGYTFGSGTRLTVV

SEQ ID NO: 72 - protein, 133 aa, synthetic construct
MGTSLLCWMALCLLGADHADTGVSQNPRHKITKRGQNVTFRCDPISEHNRLYWYRQTLGQGPEFLTYFQNEAQLEKSRLLSDRFSAERPKGSFSTLEIQRTEQGDSAMYLCASSPGTGRDTQYFGPGTRLTVL

SEQ ID NO: 73 - DNA, 387 bp, synthetic construct
  source 1..387: mol_type = other DNA
atgaagtccctgagagtgctgctggtcatcctgtggctgcagctgtcttgggtctggtcccagcagaaagaggtggaacagaacagcggccctctgtctgttcctgaaggcgctatcgcctctctgaattgcacctacagcgacagaggcagccagagcttcttctggtatcggcagtacagcggcaagagccccgagctgatcatgttcatctacagcaacggcgacaaagaggacggccggtttacagcccagctgaacaaagccagccagtacgtgtccctgctgatcagagattcccagccaagcgactccgccacctacctgtgtgccgccgacgacaagatcatcttcggcaagggaaccagactgcacatcctgcctaac

SEQ ID NO: 74 - DNA, 402 bp, synthetic construct
  source 1..402: mol_type = other DNA
atggaaaagatgctggaatgcgccttcatcgtgctgtggctgcagctgggatggctgagcggagaggaccaagtgacccagtctcccgaggccctgagactgcaggaaggcgagagcagcagcctgaattgcagctacaccgtgtccggcctgcggggcctgttctggtatagacaggaccctggcaagggccccgagttcctgtttaccctgtactctgccggcgaagagaaagaaaaagagcggctgaaggccacactgaccaagaaagagagcttcctgcacatcaccgcccccaagcctgaggacagcgccacatatctgtgcgccgtgcactctacagcccaggccggaaccgccctgatcttcggcaagggcacaaccctgtccgtgtccagcaac

SEQ ID NO: 75 - DNA, 384 bp, synthetic construct
  source 1..384: mol_type = other DNA
atgtggggcgtgttcctgctgtacgtgtccatgaagatgggcggcaccaccggccagaacatcgaccagcctaccgagatgaccgccaccgagggcgccatcgtgcagatcaattgcacctaccagaccagcggcttcaacggcctgttctggtatcagcagcacgccggcgaggcccctaccttcctgagctacaatgtgctggacggcctggaagaaaagggccggttcagcagcttcctgtccagaagcaagggctacagctacctgctgctgaaagaactgcagatgaaggacagcgcctcctacctgtgtgccgtgcggggcgatagcagctacaagctgatcttcggcagcggcacacggctgctcgtgcggcctgac

SEQ ID NO: 76 - DNA, 423 bp, synthetic construct
  source 1..423: mol_type = other DNA
attcagaaccccgatcctgccgtgtaccagctgagagacagcaagagcagcgacaagagcgtgtgtctgttcaccgacttcgacagccagaccaacgtgtcccagagcaaggacagcgacgtgtacatcaccgacaagaccgtgctggacatgcggagcatggacttcaagagcaacagcgccgtggcctggtccaacaagagcgatttcgcctgcgccaacgccttcaacaatagcattatccccgaggacacattcttccccagctccgatgtgccctgcgacgtgaagctggtggaaaagagcttcgagacagacaccaacctgaacttccagaacctgagcgtgatcggcttcagaatcctgctgctgaaggtggccggcttcaatctgctgatgaccctgagactgtggtccagctga

SEQ ID NO: 77 - DNA, 423 bp, synthetic construct
  source 1..423: mol_type = other DNA
atccagaaccccgaccccgccgtgtaccagctgagagacagcaagagcagcgacaagagcgtgtgcctgttcaccgacttcgacagccagacaaacgtgtcccagagcaaggacagcgacgtgtacatcaccgataagtgcgtgctggacatgcggagcatggacttcaagagcaacagcgccgtggcctggtccaacaagagcgatttcgcctgcgccaacgccttcaacaacagcattatccccgaggacacattcttccccagctccgacgtgccctgcgacgtgaagctggtggaaaagagcttcgagacagacaccaacctgaacttccagaatctgagcgtgatcggcttcagaatcctgctgctgaaggtggccggcttcaatctgctgatgaccctgcggctgtggtccagctga

SEQ ID NO: 78 - DNA, 420 bp, synthetic construct
  source 1..420: mol_type = other DNA
atccagaaccctgatcccgccgtgtaccagctgcgggacagcaagagcagcgacaagagcgtgtgcctgttcaccgacttcgacagccagaccaatgtgtcccagtccaaggactccgacgtgtacatcaccgataagtgcgtgctggacatgcggagcatggacttcaagagcaacagcgccgtggcctggtccaacaagagcgatttcgcctgcgccaacgccttcaacaacagcattatccccgaggacacattcttcccaagcagcgacgtgccctgcgacgtgaagctggtggaaaagtccttcgagacagacaccaacctgaatttccagaacctgagcgtgatcggcttccggattctgctgctgaaggtggccggcttcaacctgctgatgaccctgagactgtggtccagc

SEQ ID NO: 79 - DNA, 393 bp, synthetic construct
  source 1..393: mol_type = other DNA
atgggaagctggaccctgtgttgtgtgtccctgtgtatcctggtggccaagcacacagatgccggcgtgatccagtctcctagacacgaagtgaccgagatgggccaagaagtgaccctgcgctgcaagcctatcagcggccacgattacctgttctggtacagacagaccatgatgagaggcctggaactgctgatctacttcaacaacaacgtgcccatcgacgacagcggaatgcccgaggatagattcagcgccaagatgcccaacgccagcttcagcaccctgaagatccagcctagcgagcccagagatagcgccgtgtacttttgcgcctcttccagaggcggcagcggctacacatttggctctggcacaagactgaccgtggtg

SEQ ID NO: 80 - DNA, 402 bp, synthetic construct
  source 1..402: mol_type = other DNA
atgggcttccggctgctgtgttgcgtggccttctgtctgctgggagccggccctgtggatagcggcgtgacacagacacccaagcacctgatcaccgccaccggccagcgcgtgacactgagatgtagccctagaagcggcgacctgagcgtgtactggtatcagcagagcctggaccagggcctgcagttcctgatccagtactacaacggcgaggaacgggccaagggcaacatcctggaacggttcagcgcccagcagttccccgatctgcacagcgagctgaacctgagcagcctggaactgggcgacagcgccctgtacttctgtgccagcagcacccacagaggccagaccaactacggctacaccttcggcagcggcaccagactgaccgtggtg

SEQ ID NO: 81 - DNA, 399 bp, synthetic construct
  source 1..399: mol_type = other DNA
atgggcaccagcctgctgtgttggatggccctgtgtctgctgggagccgaccatgccgatacaggcgtgtcccagaacccccggcacaagatcaccaagcggggccagaacgtgaccttcagatgcgaccccatcagcgagcacaaccggctgtactggtacagacagaccctgggccagggccccgagttcctgacctacttccagaacgaggcccagctggaaaagagccggctgctgagcgacagattcagcgccgaaagacccaagggcagcttcagcaccctggaaatccagcggaccgagcagggcgacagcgccatgtatctgtgtgccagctctcccggcaccggcagagacacccagtattttggcccaggcacccggctgaccgtgctg

SEQ ID NO: 82 - protein, 195 aa, synthetic construct
EDLNKVFPPEVAVFEPSKAEIAHTQKATLVCLATGFFPDHVELSWWVNGKEVHSGVSTDPQPLKEQPGSGDKGEVPKDRFSAGSGALNDSRYCLSSRLRVSATFWQNPRNHFRCQVQFYGLSENDEWTQDRAKPVTQIVSAEAWGRADCGITSASYHQGVLSATILYEILLGKATLYAVLVSALVLMAMVKRKDF

SEQ ID NO: 83 - protein, 195 aa, synthetic construct
EDLNKVFPPEVAVFEPSKAEIAHTQKATLVCLATGFFPDHVELSWWVNGKEVHSGVSTDPQPLKEQPAGSGDKGEVPKDRFSAGSGLNDSRYCLSSRLRVSATFWQNPRNHFRCQVQFYGLSENDEWTQDRAKPVTQIVSAEAWGRADCGITSASYHQGVLSATILYEILLGKATLYAVLVSALVLMAMVKRKDF

SEQ ID NO: 84 - protein, 195 aa, synthetic construct
EDLNKVFPPEVAVFEPSKAEIAHTQKATLVCLATGFFPDHVELSWWVNGKEVHSGVSTDPQPLKEQPALGSGDKGEVPKDRFSAGSGNDSRYCLSSRLRVSATFWQNPRNHFRCQVQFYGLSENDEWTQDRAKPVTQIVSAEAWGRADCGITSASYHQGVLSATILYEILLGKATLYAVLVSALVLMAMVKRKDF

SEQ ID NO: 85 - protein, 195 aa, synthetic construct
EDLNKVFPPEVAVFEPSKAEIAHTQKATLVCLATGFFPDHVELSWWVNGKEVHSGVSTDPQPLKEQPALNDGSGDKGEVPKDRFSAGSGSRYCLSSRLRVSATFWQNPRNHFRCQVQFYGLSENDEWTQDRAKPVTQIVSAEAWGRADCGITSASYHQGVLSATILYEILLGKATLYAVLVSALVLMAMVKRKDF

SEQ ID NO: 86 - protein, 195 aa, synthetic construct
EDLNKVFPPEVAVFEPSKAEIAHTQKATLVCLATGFFPDHVELSWWVNGKEVHSGVSTDPQPLKEQPALNDSRYCLSSRLRVSATFWQNPRNHFRCQVQFYGLSENDGSGDKGEVPKDRFSAGSGEWTQDRAKPVTQIVSAEAWGRADCGITSASYHQGVLSATILYEILLGKATLYAVLVSALVLMAMVKRKDF

SEQ ID NO: 87 - protein, 195 aa, synthetic construct
EDLNKVFPPEVAVFEPSKAEIAHTQKATLVCLATGFFPDHVELSWWVNGKEVHSGVSTDPQPLKEQPALNDSRYCLSSRLRVSATFWQNPRNHFRCQVQFYGLSENDEWGSGDKGEVPKDRFSAGSGTQDRAKPVTQIVSAEAWGRADCGITSASYHQGVLSATILYEILLGKATLYAVLVSALVLMAMVKRKDF

SEQ ID NO: 88 - protein, 195 aa, synthetic construct
EDLNKVFPPEVAVFEPSKAEIAHTQKATLVCLATGFFPDHVELSWWVNGKEVHSGVSTDPQPLKEQPALNDSRYCLSSRLRVSATFWQNPRNHFRCQVQFYGLSENDEWTQDRAGSGDKGEVPKDRFSAGSGKPVTQIVSAEAWGRADCGITSASYHQGVLSATILYEILLGKATLYAVLVSALVLMAMVKRKDF

SEQ ID NO: 89 - protein, 158 aa, synthetic construct
IQNPDPAVYQLRDSKSSDKSVCLFTDFDSQTNVSQSKDSDVYITDKTVLDMRSMDFKSNSAVAWSNKSDFACANAFNNSIGSGDKGEVPKDRFSAGSGIPEDTFFPSSDVPCDVKLVEKSFETDTNLNFQNLSVIGFRILLLKVAGFNLLMTLRLWSS

SEQ ID NO: 90 - protein, 158 aa, synthetic construct
IQNPDPAVYQLRDSKSSDKSVCLFTDFDSQTNVSQSKDSDVYITDKTVLDMRSMDFKSNSAVAWSNKSDFACANAFNNSIIPGSGDKGEVPKDRFSAGSGEDTFFPSSDVPCDVKLVEKSFETDTNLNFQNLSVIGFRILLLKVAGFNLLMTLRLWSS

SEQ ID NO: 91 - protein, 158 aa, synthetic construct
IQNPDPAVYQLRDSKSSDKSVCLFTDFDSQTNVSQSKDSDVYITDKTVLDMRSMDFKSNSAVAWSNKSDFACANAFNNSIIPEDGSGDKGEVPKDRFSAGSGTFFPSSDVPCDVKLVEKSFETDTNLNFQNLSVIGFRILLLKVAGFNLLMTLRLWSS

SEQ ID NO: 92 - protein, 194 aa, synthetic construct
EDLNKVFPPEVAVFEPSKAEIAHTQKATLVCLATGFFPDHVELSWWVNGKEVHSGVSTDPQPLKEQPALNDSRYCLSSRLRVSATFWQNPRNHFRCQVQFYGLSENDEWTQDRAGSGKGEVPKDRFSAGSGKPVTQIVSAEAWGRADCGITSASYHQGVLSATILYEILLGKATLYAVLVSALVLMAMVKRKDF

SEQ ID NO: 93 - protein, 193 aa, synthetic construct
EDLNKVFPPEVAVFEPSKAEIAHTQKATLVCLATGFFPDHVELSWWVNGKEVHSGVSTDPQPLKEQPALNDSRYCLSSRLRVSATFWQNPRNHFRCQVQFYGLSENDEWTQDRAGSGGEVPKDRFSAGSGKPVTQIVSAEAWGRADCGITSASYHQGVLSATILYEILLGKATLYAVLVSALVLMAMVKRKDF

SEQ ID NO: 94 - protein, 192 aa, synthetic construct
EDLNKVFPPEVAVFEPSKAEIAHTQKATLVCLATGFFPDHVELSWWVNGKEVHSGVSTDPQPLKEQPALNDSRYCLSSRLRVSATFWQNPRNHFRCQVQFYGLSENDEWTQDRAGSGGEVPKDRFSGSGKPVTQIVSAEAWGRADCGITSASYHQGVLSATILYEILLGKATLYAVLVSALVLMAMVKRKDF

SEQ ID NO: 95 - protein, 194 aa, synthetic construct
EDLNKVFPPEVAVFEPSKAEIAHTQKATLVCLATGFFPDHVELSWWVNGKEVHSGVSTDPQPLKEQPALNDSRYCLSSRLRVSATFWQNPRNHFRCQVQFYGLSENDEWTQDRAGSGDKGEVPKDRFSGSGKPVTQIVSAEAWGRADCGITSASYHQGVLSATILYEILLGKATLYAVLVSALVLMAMVKRKDF

SEQ ID NO: 96 - protein, 192 aa, synthetic construct
EDLNKVFPPEVAVFEPSKAEIAHTQKATLVCLATGFFPDHVELSWWVNGKEVHSGVSTDPQPLKEQPALNDSRYCLSSRLRVSATFWQNPRNHFRCQVQFYGLSENDEWTQDRAGSGKGEVPKDRFGSGKPVTQIVSAEAWGRADCGITSASYHQGVLSATILYEILLGKATLYAVLVSALVLMAMVKRKDF

SEQ ID NO: 97 - protein, 192 aa, synthetic construct
EDLNKVFPPEVAVFEPSKAEIAHTQKATLVCLATGFFPDHVELSWWVNGKEVHSGVSTDPQPLKEQPGSGYPYDVPDYAGSGALNDSRYCLSSRLRVSATFWQNPRNHFRCQVQFYGLSENDEWTQDRAKPVTQIVSAEAWGRADCGITSASYHQGVLSATILYEILLGKATLYAVLVSALVLMAMVKRKDF

SEQ ID NO: 98 - protein, 192 aa, synthetic construct
EDLNKVFPPEVAVFEPSKAEIAHTQKATLVCLATGFFPDHVELSWWVNGKEVHSGVSTDPQPLKEQPAGSGYPYDVPDYAGSGLNDSRYCLSSRLRVSATFWQNPRNHFRCQVQFYGLSENDEWTQDRAKPVTQIVSAEAWGRADCGITSASYHQGVLSATILYEILLGKATLYAVLVSALVLMAMVKRKDF

SEQ ID NO: 99 - protein, 192 aa, synthetic construct
EDLNKVFPPEVAVFEPSKAEIAHTQKATLVCLATGFFPDHVELSWWVNGKEVHSGVSTDPQPLKEQPALGSGYPYDVPDYAGSGNDSRYCLSSRLRVSATFWQNPRNHFRCQVQFYGLSENDEWTQDRAKPVTQIVSAEAWGRADCGITSASYHQGVLSATILYEILLGKATLYAVLVSALVLMAMVKRKDF

SEQ ID NO: 100 - protein, 192 aa, synthetic construct
EDLNKVFPPEVAVFEPSKAEIAHTQKATLVCLATGFFPDHVELSWWVNGKEVHSGVSTDPQPLKEQPALNDGSGYPYDVPDYAGSGSRYCLSSRLRVSATFWQNPRNHFRCQVQFYGLSENDEWTQDRAKPVTQIVSAEAWGRADCGITSASYHQGVLSATILYEILLGKATLYAVLVSALVLMAMVKRKDF

SEQ ID NO: 101 - protein, 192 aa, synthetic construct
EDLNKVFPPEVAVFEPSKAEIAHTQKATLVCLATGFFPDHVELSWWVNGKEVHSGVSTDPQPLKEQPALNDSRYCLSSRLRVSATFWQNPRNHFRCQVQFYGLSENDGSGYPYDVPDYAGSGEWTQDRAKPVTQIVSAEAWGRADCGITSASYHQGVLSATILYEILLGKATLYAVLVSALVLMAMVKRKDF

SEQ ID NO: 102 - protein, 192 aa, synthetic construct
EDLNKVFPPEVAVFEPSKAEIAHTQKATLVCLATGFFPDHVELSWWVNGKEVHSGVSTDPQPLKEQPALNDSRYCLSSRLRVSATFWQNPRNHFRCQVQFYGLSENDEWGSGYPYDVPDYAGSGTQDRAKPVTQIVSAEAWGRADCGITSASYHQGVLSATILYEILLGKATLYAVLVSALVLMAMVKRKDF

SEQ ID NO: 103 - protein, 155 aa, synthetic construct
IQNPDPAVYQLRDSKSSDKSVCLFTDFDSQTNVSQSKDSDVYITDKTVLDMRSMDFKSNSAVAWSNKSDFACANAFNNSIGSGYPYDVPDYAGSGIPEDTFFPSSDVPCDVKLVEKSFETDTNLNFQNLSVIGFRILLLKVAGFNLLMTLRLWSS

SEQ ID NO: 104 - protein, 155 aa, synthetic construct
IQNPDPAVYQLRDSKSSDKSVCLFTDFDSQTNVSQSKDSDVYITDKTVLDMRSMDFKSNSAVAWSNKSDFACANAFNNSIIPGSGYPYDVPDYAGSGEDTFFPSSDVPCDVKLVEKSFETDTNLNFQNLSVIGFRILLLKVAGFNLLMTLRLWSS

SEQ ID NO: 105 - protein, 195 aa, synthetic construct
EDLNKVFPPEVAVFEPSKAEIAHTQKATLVCLATGFFPDHVELSWWVNGKEVHSGVCTDPQPLKEQPAGSGDKGEVPKDRFSAGSGLNDSRYCLSSRLRVSATFWQNPRNHFRCQVQFYGLSENDEWTQDRAKPVTQIVSAEAWGRADCGITSASYHQGVLSATILYEILLGKATLYAVLVSALVLMAMVKRKDF

SEQ ID NO: 106 - protein, 195 aa, synthetic construct
EDLNKVFPPEVAVFEPSKAEIAHTQKATLVCLATGFFPDHVELSWWVNGKEVHSGVCTDPQPLKEQPALNDSRYCLSSRLRVSATFWQNPRNHFRCQVQFYGLSENDEWTQDRAGSGDKGEVPKDRFSAGSGKPVTQIVSAEAWGRADCGITSASYHQGVLSATILYEILLGKATLYAVLVSALVLMAMVKRKDF

SEQ ID NO: 107 - protein, 196 aa, synthetic construct
EDLKNVFPPEVAVFEPSKAEIAHTQKATLVCLATGFYPDHVELSWWVNGKEVHSGVCTDPQPLKEQPAGSGDKGEVPKDRFSAGSGLNDSRYCLSSRLRVSATFWQNPRNHFRCQVQFYGLSENDEWTQDRAKPVTQIVSAEAWGRADCGITSASYHQGVLSATILYEILLGKATLYAVLVSALVLMAMVKRKDSR

SEQ ID NO: 108 - protein, 197 aa, synthetic construct
EDLKNVFPPEVAVFEPSKAEIAHTQKATLVCLATGFYPDHVELSWWVNGKEVHSGVCTDPQPLKEQPALNDSRYCLSSRLRVSATFWQNPRNHFRCQVQFYGLSENDEWTQDRAGSGDKGEVPKDRFSAGSGKPVTQIVSAEAWGRADCGITSASYHQGVLSATILYEILLGKATLYAVLVSALVLMAMVKRKDSRG

SEQ ID NO: 109 - protein, 9 aa, synthetic construct
YLNMWITTC

SEQ ID NO: 110 - protein, 9 aa, synthetic construct
ICLQWITQC

SEQ ID NO: 111 - protein, 9 aa, synthetic construct
SLLFWILIC

SEQ ID NO: 112 - protein, 9 aa, synthetic construct
SLCMVITIY

SEQ ID NO: 113 - protein, 9 aa, synthetic construct
SLLLWPTRL

SEQ ID NO: 114 - protein, 9 aa, synthetic construct
GLLNWITGA

SEQ ID NO: 115 - protein, 9 aa, synthetic construct
SLLMSIHNI

SEQ ID NO: 116 - protein, 9 aa, synthetic construct
SLLMTISLL

SEQ ID NO: 117 - protein, 9 aa, synthetic construct
SILMYITSL

SEQ ID NO: 118 - protein, 9 aa, synthetic construct
SLLQWVTSR

SEQ ID NO: 119 - protein, 9 aa, synthetic construct
SLLMWMLRL

SEQ ID NO: 120 - protein, 9 aa, synthetic construct
PLLVWITTL

SEQ ID NO: 121 - protein, 9 aa, synthetic construct
LLLMIITFW

SEQ ID NO: 122 - protein, 9 aa, synthetic construct
SLLYVIHTC

SEQ ID NO: 123 - protein, 9 aa, synthetic construct
YLLYGITHC

SEQ ID NO: 124 - protein, 9 aa, synthetic construct
SLMYWITIQ

SEQ ID NO: 125 - protein, 9 aa, synthetic construct
NLLFWICGC

SEQ ID NO: 126 - protein, 9 aa, synthetic construct
NLKMWIQEC

SEQ ID NO: 127 - protein, 9 aa, synthetic construct
YLKMSIAQC

SEQ ID NO: 128 - protein, 9 aa, synthetic construct
SLLCYIKHC

SEQ ID NO: 129 - protein, 9 aa, synthetic construct
SLQMGYTQG

SEQ ID NO: 130 - protein, 9 aa, synthetic construct
SLLSSVTQG

SEQ ID NO: 131 - protein, 9 aa, synthetic construct
SLLSHITSS

SEQ ID NO: 132 - protein, 9 aa, synthetic construct
SLLMLIAMS

SEQ ID NO: 133 - protein, 9 aa, synthetic construct
SLDMWRLGC

SEQ ID NO: 134 - protein, 9 aa, synthetic construct
SILVWTTQP

SEQ ID NO: 135 - protein, 9 aa, synthetic construct
SLLMKIFHS

SEQ ID NO: 136 - protein, 9 aa, synthetic construct
SLLSKITFD

SEQ ID NO: 137 - protein, 9 aa, synthetic construct
SLLEVLTQD

SEQ ID NO: 138 - protein, 9 aa, synthetic construct
ELLMWPLQE

SEQ ID NO: 139 - protein, 9 aa, synthetic construct
GLLQWITNL

SEQ ID NO: 140 - protein, 9 aa, synthetic construct
SLLMPWTSL

SEQ ID NO: 141 - protein, 177 aa, synthetic construct
EDLNKVFPPEVAVFEPSKAEIAHTQKATLVCLATGFFPDHVELSWWVNGKEVHSGVSTDPQPLKEQPALNDSRYCLSSRLRVSATFWQNPRNHFRCQVQFYGLSENDEWTQDRAKPVTQIVSAEAWGRADCGITSASYHQGVLSATILYEILLGKATLYAVLVSALVLMAMVKRKDF

SEQ ID NO: 142 - DNA, 531 bp, synthetic construct
  source 1..531: mol_type = other DNA
gaagatctgaacaaggtgttccctccagaggtggccgtgttcgagccttctaaggccgagattgcccacacacagaaagccacactcgtgtgcctggctaccggcttctttcctgaccacgtggaactgtcttggtgggtcaacggcaaagaggtgcacagcggcgtcagcacagatccccagcctctgaaagaacagcccgctctgaacgacagccggtactgtctgagcagcagactgagagtgtccgccacattctggcagaaccccagaaaccacttcagatgccaggtgcagttctacggcctgagcgagaacgatgagtggacccaggatagagccaagcctgtgacacagatcgtgtctgccgaagcctggggcagagccgattgtggaattaccagcgccagctaccatcagggcgtgctgtctgccacaatcctgtacgagatcctgctgggcaaagccactctgtacgccgtgctggtgtctgccctggtgctgatggccatggtcaagagaaaggacttt

SEQ ID NO: 143 - protein, 269 aa, synthetic construct
MKSLRVLLVILWLQLSWVWSQQKEVEQNSGPLSVPEGAIASLNCTYSDRGSQSFFWYRQYSGKSPELIMFIYSNGDKEDGRFTAQLNKASQYVSLLIRDSQPSDSATYLCAADDKIIFGKGTRLHILPNIQNPDPAVYQLRDSKSSDKSVCLFTDFDSQTNVSQSKDSDVYITDKTVLDMRSMDFKSNSAVAWSNKSDFACANAFNNSIIPEDTFFPSSDVPCDVKLVEKSFETDTNLNFQNLSVIGFRILLLKVAGFNLLMTLRLWSS

SEQ ID NO: 144 - protein, 308 aa, synthetic construct
MGSWTLCCVSLCILVAKHTDAGVIQSPRHEVTEMGQEVTLRCKPISGHDYLFWYRQTMMRGLELLIYFNNNVPIDDSGMPEDRFSAKMPNASFSTLKIQPSEPRDSAVYFCASSRGGSGYTFGSGTRLTVVEDLNKVFPPEVAVFEPSKAEIAHTQKATLVCLATGFFPDHVELSWWVNGKEVHSGVSTDPQPLKEQPALNDSRYCLSSRLRVSATFWQNPRNHFRCQVQFYGLSENDEWTQDRAKPVTQIVSAEAWGRADCGITSASYHQGVLSATILYEILLGKATLYAVLVSALVLMAMVKRKDF

SEQ ID NO: 145 - protein, 14 aa, synthetic construct
FNNSIIPEDTFFPS

SEQ ID NO: 146 - protein, 15 aa, synthetic construct
DPQPLKEQPALNDSR

SEQ ID NO: 147 - protein, 18 aa, synthetic construct
YGLSENDEWTQDRAKPVT

SEQ ID NO: 148 - protein, 20 aa, synthetic construct
FKSNSAVAWSNKSDFACANA

SEQ ID NO: 149 - protein, 20 aa, synthetic construct
SDVPCDVKLVEKSFETDTNL

SEQ ID NO: 150 - protein, 20 aa, synthetic construct
DHVELSWWVNGKEVHSGVST

SEQ ID NO: 151 - protein, 20 aa, synthetic construct
YCLSSRLRVSATFWQNPRNH

SEQ ID NO: 152 - protein, 20 aa, synthetic construct
RVSATFWQNPRNHFRCQVQF

SEQ ID NO: 153 - protein, 20 aa, synthetic construct
QIVSAEAWGRADCGITSASY

SEQ ID NO: 154 - protein, 6 aa, synthetic construct
EVPKDR

SEQ ID NO: 155 - protein, 20 aa, synthetic construct
WVNGKEVHSGVSTDPQPLKE

SEQ ID NO: 156 - protein, 20 aa, synthetic construct
FWQNPRNHFRCQVQFYGLSE

SEQ ID NO: 157 - protein, 20 aa, synthetic construct
NPRNHFRCQVQFYGLSENDE

SEQ ID NO: 158 - protein, 20 aa, synthetic construct
HFRCQVQFYGLSENDEWTQD

SEQ ID NO: 159 - protein, 20 aa, synthetic construct
QPALNDSRYCLSSRLRVSAT

SEQ ID NO: 160 - protein, 20 aa, synthetic construct
NDEWTQDRAKPVTQIVSAEA

SEQ ID NO: 161 - protein, 20 aa, synthetic construct
WTQDRAKPVTQIVSAEAWGR

SEQ ID NO: 162 - protein, 20 aa, synthetic construct
RAKPVTQIVSAEAWGRADCG

SEQ ID NO: 163 - protein, 12 aa, synthetic construct
GSGEVPKDRGSG